European Patent Application EP 4 674 427 A1, published January 7, 2026. Title: 一种治疗或改善恶病质的方法. Applicant: 周云夫. The sequence listing filed with the application follows.

SEQUENCE LISTING (8 sequences)

SEQ ID NO: 1 - protein, 459 aa, synthetic construct
MPTSVPRGAPFLLLPPLLMLSAVLAVPVDRAAPPQEDSQATETPDTGLYYHRYLQEVINVLETDGHFREKLQAANAEDIKSGKLSQELDFVSHNVRTKLDELKRQEVSRLRMLLKAKMDAKQEPNLQVDHMNLLKQFEHLDPQNQHTFEARDLELLIQTATRDLAQYDAAHHEEFKRYEMLKEHERRRYLESLGEEQRKEAERKLQEQQRRHREHPKVNVPGSQAQLKEVWEELDGLDPNRFNPKTFFILHDINSDGVLDEQELEALFTKELEKVYDPKNEEDDMREMEEERLRMREHVMKNVDTNQDRLVTLEEFLASTQRKEFGDTGEGWKTVEMSPAYTEEELKRFEEELAAREAELNARAQRLSQETEALGRSQDRLEAQKRELQQAVLQMEQRKQQLQEQSAPPSKPDGQLQFRADTDDAPVPAPAGDQKDVPASEKKVPEQPPELPQLDSQHL

SEQ ID NO: 2 - protein, 461 aa, synthetic construct
MPPSGPRGTLLLLPLLLLLLLRAVLAVPLERGAPNKEETPATESPDTGLYYHRYLQEVIDVLETDGHFREKLQAANAEDIKSGKLSRELDFVSHHVRTKLDELKRQEVSRLRMLLKAKMDAEQDPNVQVDHLNLLKQFEHLDPQNQHTFEARDLELLIQTATRDLAQYDAAHHEEFKRYEMLKEHERRRYLESLGEEQRKEAERKLEEQQRRHREHPKVNVPGSQAQLKEVWEELDGLDPNRFNPKTFFILHDINSDGVLDEQELEALFTKELEKVYDPKNEEDDMREMEEERLRMREHVMKNVDTNQDRLVTLEEFLASTQRKEFGDTGEGWETVEMHPAYTEEELRRFEEELAAREAELNAKAQRLSQETEALGRSQGRLEAQKRELQQAVLHMEQRKQQQQQQQGHKAPAAHPEGQLKFHPDTDDVPVPAPAGDQKEVDTSEKKLLERLPEVEVPQHL

SEQ ID NO: 3 - protein, 420 aa, synthetic construct
MRWRIIQVQYCFLLVPCMLTALEAVPIDVDKTKVHNTEPVENARIEPPDTGLYYDEYLKQVIEVLETDPHFREKLQKADIEEIRSGRLSQELDLVSHKVRTRLDELKRQEVGRLRMLIKAKLDALQDTGMNHHLLLKQFEHLNHQNPNTFESRDLDMLIKAATADLEQYDRTRHEEFKKYEMMKEHERREYLKTLSEEKRKEEESKFEEMKRKHEDHPKVNHPGSKDQLKEVWEETDGLDPNDFDPKTFFKLHDVNNDGFLDEQELEALFTRELEKVYNPQNAEDDMIEMEEERLRMREHVMSEIDNNKDRLVTLEEFLRATEKKEFLEPDSWETLDQQQLFTEDELKEYESIIAIQENELKKRAEELQKQKEDLQRQHDHLEAQKQEYHQAVQHLEQKKLQQGIAPSGPAGELKFEPHT

SEQ ID NO: 4 - protein, 420 aa, synthetic construct
MRWRTILLQYCFLLITCLLTALEAVPIDIDKTKVQNIHPVESAKIEPPDTGLYYDEYLKQVIDVLETDKHFREKLQKADIEEIKSGRLSKELDLVSHHVRTKLDELKRQEVGRLRMLIKAKLDSLQDIGMDHQALLKQFDHLNHLNPDKFESTDLDMLIKAATSDLEHYDKTRHEEFKKYEMMKEHERREYLKTLNEEKRKEEESKFEEMKKKHENHPKVNHPGSKDQLKEVWEETDGLDPNDFDPKTFFKLHDVNSDGFLDEQELEALFTKELEKVYDPKNEEDDMVEMEEERLRMREHVMNEVDTNKDRLVTLEEFLKATEKKEFLEPDSWETLDQQQFFTEEELKEYENIIALQENELKKKADELQKQKEELQRQHDQLEAQKLEYHQVIQQMEQKKLQQGIPPSGPAGELKFEPHI

SEQ ID NO: 5 - DNA, 1380 bp, synthetic construct
  source 1..1380: mol_type = other DNA
atgcctacctcggtgccccgcggggccccttttcttctcctaccacctctactgatgctgtctgctgtgctggcagtgcccgtggaccgcgcagcacctcctcaggaggacagccaggccactgagaccccggacacgggcctgtactaccaccggtacctccaggaggtcatcaacgtgctagagacagatgggcacttccgggagaagctgcaggctgccaacgctgaggacattaagagtggaaagctgagccaagagctggacttcgtcagccacaacgtccgaaccaagctggatgagctcaagcgacaggaggtgtcgaggctgcggatgctgctcaaggccaagatggatgcaaagcaggagcccaacttgcaggtggaccacatgaacctcctgaagcagtttgagcacctggaccctcagaaccagcacacgtttgaggctcgggacctagagctgctgatccagacggccacccgagacctcgcccagtatgacgctgcacaccatgaagagttcaaacgctacgagatgctcaaggaacatgagaggagacgatacctggagtctctgggagaggagcagcggaaggaggccgagaggaagctccaagagcaacagcgcagacaccgggaacaccccaaagtcaatgttcctggcagccaagcccagttgaaggaggtgtgggaggagttggatggattggaccccaacaggttcaaccccaagaccttcttcatactgcatgacatcaacagtgatggtgtcctagatgagcaagaactggaagctctctttaccaaggagctggagaaggtgtatgacccgaagaatgaggaggatgacatgagagagatggaggaagaacggcttcgcatgcgggagcacgtgatgaagaatgtggacaccaaccaggaccggcttgtgaccctggaggagttcctggcatccacccagaggaaggagttcggggacactggggaggggtggaagacagtggaaatgtccccagcctacacagaggaggagctgaagcgttttgaagaggagctggctgcccgggaagctgagctgaatgccagggcccagcgcctcagccaggagacagaggccctggggcgctcccaggaccgcctggaggcacagaagagagagctgcagcaggctgttctgcagatggagcagaggaagcagcaactgcaagaacagagcgctccgccttccaaacctgacgggcagctgcagttccgtgcagacacagatgacgctcctgtcccagctccagcaggtgaccagaaagatgtgcctgcttctgagaagaaggtcccagagcagccccctgagctgccacagctggattcccagcatttataa

SEQ ID NO: 6 - DNA, 1386 bp, synthetic construct
  source 1..1386: mol_type = other DNA
atgcctccctctgggccccgaggaaccctccttctgttgccgctgctgctgctgctcctgcttcgcgccgtgctggctgtccccctggagcgaggggcgcccaacaaggaggagacccctgcgactgagagtcccgacacaggcctgtactaccaccggtacctccaggaggtcatcgatgtactggagacggatgggcatttccgagagaagctgcaggctgccaatgcggaggacatcaagagcgggaagctgagccgagagctggactttgtcagccaccacgtccgcaccaagctggatgagctcaagcgacaggaggtgtcacggctgcggatgctgctcaaggccaagatggacgccgagcaggatcccaatgtacaggtggatcatctgaatctcctgaaacagtttgaacacctggaccctcagaaccagcatacattcgaggcccgcgacctggagctgctgatccagacggccacccgggaccttgcccagtacgacgcagcccatcatgaagagttcaagcgctacgagatgcttaaggaacacgagagacggcgttatctggagtcactgggagaggagcagagaaaggaggcggagaggaagctggaagagcaacagcgccggcaccgcgagcaccctaaagtcaacgtgcctggcagccaagcccagttgaaggaggtgtgggaggagctggatggactggaccccaacaggtttaaccccaagaccttcttcatactgcatgatatcaacagtgatggtgtcctggatgagcaggagctggaggcactcttcaccaaggagctggagaaagtgtacgacccaaagaatgaggaggacgacatgcgggagatggaggaggagcgactgcgcatgcgggagcatgtgatgaagaatgtggacaccaaccaggaccgcctcgtgaccctggaggagttcctcgcatccactcagaggaaggagtttggggacaccggggagggctgggagacagtggagatgcaccctgcctacaccgaggaagagctgaggcgctttgaagaggagctggctgcccgggaggcagagctgaatgccaaggcccagcgcctcagccaggagacagaggctctagggcggtcccagggccgcctggaggcccagaagagagagctgcagcaggctgtgctgcacatggagcagcggaagcagcagcagcagcagcagcaaggccacaaggccccggctgcccaccctgaggggcagctcaagttccacccagacacagacgatgtacctgtcccagctccagccggtgaccagaaggaggtggacacttcagaaaagaaacttctcgagcggctccctgaggttgaggtgccccagcatctgtga

SEQ ID NO: 7 - DNA, 1263 bp, synthetic construct
  source 1..1263: mol_type = other DNA
atgaggtggaggatcatccaagtacagtactgttttctcttggttccgtgcatgctgaccgctctggaagctgttcctatcgatgtggacaagaccaaagtacacaacactgagccagtggaaaatgcaaggatagagccaccagatactggactttattatgatgaatacctcaagcaagtgattgaagtcttggaaacagatccacatttcagagaaaagctccagaaagcagacatagaggagataaggagcgggaggctgagtcaagagctggacttagtaagtcacaaagtgaggacgagactggatgagctgaagaggcaagaagtaggaagactgcggatgctcatcaaagctaagctggatgcccttcaagacactggcatgaatcaccaccttcttctgaagcagtttgaacacctgaaccaccagaatcctaacacatttgaatccagagatttggatatgctaatcaaagcagctaccgcggatctggagcaatatgaccggactcggcatgaagagtttaagaagtacgagatgatgaaggaacacgagcggagagagtatttaaaaacgctgagtgaggagaagaggaaagaagaagagtctaagtttgaagagatgaagaggaagcacgaagaccaccccaaagttaatcatcccggaagcaaagatcaactaaaagaggtttgggaagagactgatggattggaccctaatgactttgaccccaagacatttttcaaattacatgatgttaacaacgatggattcctggatgaacaagaattagaagcactattcacaagagagttggagaaagtgtataacccacaaaatgcagaggacgatatgatagaaatggaagaggagaggctcaggatgagagaacacgtcatgagtgagattgataacaacaaagaccgattggtgactctggaggaattcctgagagctacagagaagaaagaattcctggagcctgatagctgggagacactggaccagcaacagttattcaccgaggacgagcttaaagagtatgaaagcattattgctatccaagagaacgagcttaagaagagggcggaagagctgcagaaacagaaggaggatctgcagcggcagcacgaccacctcgaggcgcagaagcaggagtatcatcaggccgtccagcacctggaacagaagaaacttcaacaaggcattgctccatcagggccagcgggagagctgaagtttgagccacacacataa

SEQ ID NO: 8 - DNA, 1266 bp, synthetic construct
  source 1..1266: mol_type = other DNA
atgatgaggtggaggaccatcctgctacagtattgctttctcttgattacatgtttacttactgctcttgaagctgtgcctattgacatagacaagacaaaagtacaaaatattcaccctgtggaaagtgcgaagatagaaccaccagatactggactttattatgatgaatatctcaagcaagtgattgatgtgctggaaacagataaacacttcagagaaaagctccagaaagcagacatagaggaaataaagagtgggaggctaagcaaagaactggatttagtaagtcaccatgtgaggacaaaacttgatgaactgaaaaggcaagaagtaggaaggttaagaatgttaattaaagctaagttggattcccttcaagatataggcatggaccaccaagctcttctaaaacaatttgatcacctaaaccacctgaatcctgacaagtttgaatccacagatttagatatgctaatcaaagcggcaacaagtgatctggaacactatgacaagactcgtcatgaagaatttaaaaaatatgaaatgatgaaggaacatgaaaggagagaatatttaaaaacattgaatgaagaaaagagaaaagaagaagagtctaaatttgaagaaatgaagaaaaagcatgaaaatcaccctaaagttaatcacccaggaagcaaagatcaactaaaagaggtatgggaagagactgatggattggatcctaatgactttgaccccaagacatttttcaaattacatgatgtcaatagtgatggattcctggatgaacaagaattagaagccctatttactaaagagttggagaaagtatatgaccctaaaaatgaagaggatgatatggtagaaatggaagaagaaaggcttagaatgagggaacatgtaatgaatgaggttgatactaacaaagacagattggtgactctggaggagtttttgaaagccacagaaaaaaaagaattcttggagccagatagctgggagacattagatcagcaacagttcttcacagaggaagaactaaaagaatatgaaaatattattgctttacaagaaaatgaacttaagaagaaggcagatgagcttcagaaacaaaaagaagagctacaacgtcagcatgatcaactggaggctcagaagctggaatatcatcaggtcatacagcagatggaacaaaaaaaattacaacaaggaattcctccatcagggccagctggagaattgaagtttgagccacacatttaa